European Patent Application EP 4 137 514 A1, published February 22, 2023. Title: METHODS OF TREATING PSORIASIS USING IL-17 BINDING MOLECULES. Applicant: Novartis AG. Application EP. The sequence listing filed with the application follows.

SEQUENCE LISTING (21 sequences)

SEQ ID NO: 1 - protein, 5 aa, synthetic construct
  REGION 1..5: note = CDR1 = hypervariable region 1 of heavy chain of AIN457
NYWMN

SEQ ID NO: 2 - protein, 17 aa, synthetic construct
  REGION 1..17: note = CDR2 = hypervariable region 2 of heavy chain of AIN457
AINQDGSEKYYVGSVKG

SEQ ID NO: 3 - protein, 18 aa, synthetic construct
  REGION 1..18: note = CDR3 = hypervariable region 3 of heavy chain of AIN457
DYYDILTDYYIHYWYFDL

SEQ ID NO: 4 - protein, 12 aa, synthetic construct
  REGION 1..12: note = CDR1' = hypervariable region 1 of light chain of AIN457
RASQSVSSSYLA

SEQ ID NO: 5 - protein, 7 aa, synthetic construct
  REGION 1..7: note = CDR2' = hypervariable region 2 of light chain AIN457
GASSRAT

SEQ ID NO: 6 - protein, 9 aa, synthetic construct
  REGION 1..9: note = CDR3' = hypervariable region 3 of light chain AIN457
QQYGSSPCT

SEQ ID NO: 7 - DNA, 381 bp, Homo sapiens
  source 1..381: mol_type = unassigned DNA
  CDS 1..381: protein_id = 18; transl_table = 1
gaggtgcagttggtggagtctgggggaggcttggtccagcctggggggtccctgagactctcctgtgcagcctctggattcacctttagtaactattggatgaactgggtccgccaggctccagggaaagggctggagtgggtggccgccataaaccaagatggaagtgagaaatactatgtgggctctgtgaagggccgattcaccatctccagagacaacgccaagaactcactgtatctgcaaatgaacagcctgagagtcgaggacacggctgtgtattactgtgtgagggactattacgatattttgaccgattattacatccactattggtacttcgatctctggggccgtggcaccctggtcactgtctcctca

SEQ ID NO: 8 - protein, 127 aa, Homo sapiens [sequence omitted]

SEQ ID NO: 9 - DNA, 327 bp, Homo sapiens
  source 1..327: mol_type = unassigned DNA
  CDS 1..327: protein_id = 19; transl_table = 1; translation = EIVLTQSPGTLSLSPGERATLSCRASQSVSSSYLAWYQQKPGQAPRLLIYGASSRATGIPDRFSGSGSGTDFTLTISRLEPEDFAVYYCQQYGSSPCTFGQGTRLEIKR
gaaattgtgttgacgcagtctccaggcaccctgtctttgtctccaggggaaagagccaccctctcctgcagggccagtcagagtgttagcagcagctacttagcctggtaccagcagaaacctggccaggctcccaggctcctcatctatggtgcatccagcagggccactggcatcccagacaggttcagtggcagtgggtctgggacagacttcactctcaccatcagcagactggagcctgaagattttgcagtgtattactgtcagcagtatggtagctcaccgtgcaccttcggccaagggacacgactggagattaaacga

SEQ ID NO: 10 - protein, 109 aa, Homo sapiens
EIVLTQSPGTLSLSPGERATLSCRASQSVSSSYLAWYQQKPGQAPRLLIYGASSRATGIPDRFSGSGSGTDFTLTISRLEPEDFAVYYCQQYGSSPCTFGQGTRLEIKR

SEQ ID NO: 11 - protein, 10 aa, synthetic construct
  REGION 1..10: note = CDR1-x = hypervariable domain x of heavy chain of AIN457
GFTFSNYWMN

SEQ ID NO: 12 - protein, 11 aa, synthetic construct
  REGION 1..11: note = CDR2-x = hypervariable domain of heavy chain x of AIN457
AINQDGSEKYY

SEQ ID NO: 13 - protein, 23 aa, synthetic construct
  REGION 1..23: note = CDR3-x = hypervariable domain x of heavy chain AIN457
CVRDYYDILTDYYIHYWYFDLWG

SEQ ID NO: 14 - DNA, 711 bp, Homo sapiens
  source 1..711: mol_type = unassigned DNA
  CDS 1..711: protein_id = 20; translation = TMETPAELLFLLLLWLPDTTGEIVLTQSPGTLSLSPGERATLSCRASQSVSSSYLAWYQQKPGQAPRLLIYGASSRATGIPDRFSGSGSGTDFTLTISRLEPEDFAVYYCQQYGSSPCTFGQGTRLEIKRTVAAPSVFIFPPSDEQLKSGTASVVCLLNNFYPREAKVQWKVDNALQSGNSQESVTEQDSKDSTYSLSSTLTLSKADYEKHKVYACEVTHQGLSSPVTKSFNRGEC
accatggaaaccccagcggagcttctcttcctcctgctactctggctcccagataccaccggagaaattgtgttgacgcagtctccaggcaccctgtctttgtctccaggggaaagagccaccctctcctgcagggccagtcagagtgttagcagcagctacttagcctggtaccagcagaaacctggccaggctcccaggctcctcatctatggtgcatccagcagggccactggcatcccagacaggttcagtggcagtgggtctgggacagacttcactctcaccatcagcagactggagcctgaagattttgcagtgtattactgtcagcagtatggtagctcaccgtgcaccttcggccaagggacacgactggagattaaacgaactgtggctgcaccatctgtcttcatcttcccgccatctgatgagcagttgaaatctggaactgcctctgttgtgtgcctgctgaataacttctatcccagagaggccaaagtacagtggaaggtggataacgccctccaatcgggtaactcccaggagagtgtcacagagcaggacagcaaggacagcacctacagcctcagcagcaccctgacgctgagcaaagcagactacgagaaacacaaagtctacgcctgcgaagtcacccatcagggcctgagctcgcccgtcacaaagagcttcaacaggggagagtgttag

SEQ ID NO: 15 - protein, 236 aa, Homo sapiens
TMETPAELLFLLLLWLPDTTGEIVLTQSPGTLSLSPGERATLSCRASQSVSSSYLAWYQQKPGQAPRLLIYGASSRATGIPDRFSGSGSGTDFTLTISRLEPEDFAVYYCQQYGSSPCTFGQGTRLEIKRTVAAPSVFIFPPSDEQLKSGTASVVCLLNNFYPREAKVQWKVDNALQSGNSQESVTEQDSKDSTYSLSSTLTLSKADYEKHKVYACEVTHQGLSSPVTKSFNRGEC

SEQ ID NO: 16 - DNA, 783 bp, Homo sapiens
  source 1..783: mol_type = unassigned DNA
  CDS 1..783: protein_id = 21; transl_table = 1
accatggaattggggctgagctgggttttccttgttgctattttagaaggtgtccactgtgaggtgcagttggtggagtctgggggaggcttggtccagcctggggggtccctgagactctcctgtgcagcctctggattcacctttagtaactattggatgaactgggtccgccaggctccagggaaagggctggagtgggtggccgccataaaccaagatggaagtgagaaatactatgtgggctctgtgaagggccgattcaccatctccagagacaacgccaagaactcactgtatctgcaaatgaacagcctgagagtcgaggacacggctgtgtattactgtgtgagggactattacgatattttgaccgattattacatccactattggtacttcgatctctggggccgtggcaccctggtcactgtctcctcagcctccaccaagggcccatcggtcttccccctggcaccctcctccaagagcacctctgggggcacagcggccctgggctgcctggtcaaggactacttccccgaaccggtgacggtgtcgtggaactcaggcgccctgaccagcggcgtgcacaccttcccggctgtcctacagtcctcaggactctactccctcagcagcgtggtgaccgtgccctccagcagcttgggcacccagacctacatctgcaacgtgaatcacaagcccagcaacaccaaggtggacaagagagttgagcccaaatcttgtgacaaaactcacacatgcccaccgtgcccataa

SEQ ID NO: 17 - protein, 260 aa, Homo sapiens
TMELGLSWVFLVAILEGVHCEVQLVESGGGLVQPGGSLRLSCAASGFTFSNYWMNWVRQAPGKGLEWVAAINQDGSEKYYVGSVKGRFTISRDNAKNSLYLQMNSLRVEDTAVYYCVRDYYDILTDYYIHYWYFDLWGRGTLVTVSSASTKGPSVFPLAPSSKSTSGGTAALGCLVKDYFPEPVTVSWNSGALTSGVHTFPAVLQSSGLYSLSSVVTVPSSSLGTQTYICNVNHKPSNTKVDKRVEPKSCDKTHTCPPCP

SEQ ID NO: 18 - protein, 127 aa, Homo sapiens [sequence omitted]

SEQ ID NO: 19 - protein, 109 aa, Homo sapiens; identical to SEQ ID NO: 10

SEQ ID NO: 20 - protein, 236 aa, Homo sapiens; identical to SEQ ID NO: 15

SEQ ID NO: 21 - protein, 260 aa, Homo sapiens; identical to SEQ ID NO: 17